European Patent Specification EP 3 601 325 B1, published July 19, 2023. Title: NEW TAU SPECIES. Applicant: INSERM. The sequence listing filed with the application follows.

SEQUENCE LISTING (14 sequences)

SEQ ID NO: 1 - protein, 342 aa, Homo sapiens [sequence omitted]

SEQ ID NO: 2 - protein, 371 aa, Homo sapiens [sequence omitted]

SEQ ID NO: 3 - protein, 373 aa, Homo sapiens
  MOD_RES (1)..(1): ACETYLATION
MEDHAGTYGLGDRKDQGGYTMHQDQEGDTDAGLKAEEAGIGDTPSLEDEAAGHVTQARMVSKSKDGTGSDDKKAKGADGKTKIATPRGAAPPGQKGQANATRIPAKTPPAPKTPPSSGEPPKSGDRSGYSSPGSPGTPGSRSRTPSLPTPPTREPKKVAVVRTPPKSPSSAKSRLQTAPVPMPDLKNVKSKIGSTENLKHQPGGGKVQIINKKLDLSNVQSKCGSKDNIKHVPGGGSVQIVYKPVDLSKVTSKCGSLGNIHHKPGGGQVEVKSEKLDFKDRVQSKIGSLDNITHVPGGGNKKIETHKLTFRENAKAKTDHGAEIVYKSPVVSGDTSPRHLSNVSSTGSIDMVDSPQLATLADEVSASLAKQGL

SEQ ID NO: 4 - protein, 400 aa, Homo sapiens
  MOD_RES (1)..(1): ACETYLATION
MEDHAGTYGLGDRKDQGGYTMHQDQEGDTDAGLKESPLQTPTEDGSEEPGSETSDAKSTPTAEDVTAPLVDEGAPGKQAAAQPHTEIPEGTTAEEAGIGDTPSLEDEAAGHVTQARMVSKSKDGTGSDDKKAKGADGKTKIATPRGAAPPGQKGQANATRIPAKTPPAPKTPPSSGEPPKSGDRSGYSSPGSPGTPGSRSRTPSLPTPPTREPKKVAVVRTPPKSPSSAKSRLQTAPVPMPDLKNVKSKIGSTENLKHQPGGGKVQIVYKPVDLSKVTSKCGSLGNIHHKPGGGQVEVKSEKLDFKDRVQSKIGSLDNITHVPGGGNKKIETHKLTFRENAKAKTDHGAEIVYKSPVVSGDTSPRHLSNVSSTGSIDMVDSPQLATLADEVSASLAKQGL

SEQ ID NO: 5 - protein, 402 aa, Homo sapiens
  MOD_RES (1)..(1): ACETYLATION
MEDHAGTYGLGDRKDQGGYTMHQDQEGDTDAGLKESPLQTPTEDGSEEPGSETSDAKSTPTAEAEEAGIGDTPSLEDEAAGHVTQARMVSKSKDGTGSDDKKAKGADGKTKIATPRGAAPPGQKGQANATRIPAKTPPAPKTPPSSGEPPKSGDRSGYSSPGSPGTPGSRSRTPSLPTPPTREPKKVAVVRTPPKSPSSAKSRLQTAPVPMPDLKNVKSKIGSTENLKHQPGGGKVQIINKKLDLSNVQSKCGSKDNIKHVPGGGSVQIVYKPVDLSKVTSKCGSLGNIHHKPGGGQVEVKSEKLDFKDRVQSKIGSLDNITHVPGGGNKKIETHKLTFRENAKAKTDHGAEIVYKSPVVSGDTSPRHLSNVSSTGSIDMVDSPQLATLADEVSASLAKQGL

SEQ ID NO: 6 - protein, 431 aa, Homo sapiens
  MOD_RES (1)..(1): ACETYLATION
MEDHAGTYGLGDRKDQGGYTMHQDQEGDTDAGLKESPLQTPTEDGSEEPGSETSDAKSTPTAEDVTAPLVDEGAPGKQAAAQPHTEIPEGTTAEEAGIGDTPSLEDEAAGHVTQARMVSKSKDGTGSDDKKAKGADGKTKIATPRGAAPPGQKGQANATRIPAKTPPAPKTPPSSGEPPKSGDRSGYSSPGSPGTPGSRSRTPSLPTPPTREPKKVAVVRTPPKSPSSAKSRLQTAPVPMPDLKNVKSKIGSTENLKHQPGGGKVQIINKKLDLSNVQSKCGSKDNIKHVPGGGSVQIVYKPVDLSKVTSKCGSLGNIHHKPGGGQVEVKSEKLDFKDRVQSKIGSLDNITHVPGGGNKKIETHKLTFRENAKAKTDHGAEIVYKSPVVSGDTSPRHLSNVSSTGSIDMVDSPQLATLADEVSASLAKQGL

SEQ ID NO: 7 - protein, 766 aa, Homo sapiens
  MOD_RES (1)..(1): ACETYLATION
MEDHAGTYGLGDRKDQGGYTMHQDQEGDTDAGLKESPLQTPTEDGSEEPGSETSDAKSTPTAEDVTAPLVDEGAPGKQAAAQPHTEIPEGTTAEEAGIGDTPSLEDEAAGHVTQEPESGKVVQEGFLREPGPPGLSHQLMSGMPGAPLLPEGPREATRQPSGTGPEDTEGGRHAPELLKHQLLGDLHQEGPPLKGAGGKERPGSKEEVDEDRDVDESSPQDSPPSKASPAQDGRPPQTAAREATSIPGFPAEGAIPLPVDFLSKVSTEIPASEPDGPSVGRAKGQDAPLEFTFHVEITPNVQKEQAHSEEHLGRAAFPGAPGEGPEARGPSLGEDTKEADLPEPSEKQPAAAPRGKPVSRVPQLKARMVSKSKDGTGSDDKKAKTSTRSSAKTLKNRPCLSPKHPTPGSSDPLIQPSSPAVCPEPPSSPKYVSSVTSRTGSSGAKEMKLKGADGKTKIATPRGAAPPGQKGQANATRIPAKTPPAPKTPPSSATKQVQRRPPPAGPRSERGEPPKSGDRSGYSSPGSPGTPGSRSRTPSLPTPPTREPKKVAVVRTPPKSPSSAKSRLQTAPVPMPDLKNVKSKIGSTENLKHQPGGGKVQIINKKLDLSNVQSKCGSKDNIKHVPGGGSVQIVYKPVDLSKVTSKCGSLGNIHHKPGGGQVEVKSEKLDFKDRVQSKIGSLDNITHVPGGGNKKIETHKLTFRENAKAKTDHGAEIVYKSPVVSGDTSPRHLSNVSSTGSIDMVDSPQLATLADEVSASLAKQGL

SEQ ID NO: 8 - protein, 11 aa, Artificial
  Tau N-Alpha Acetyl-Met11-21 (antigen)
  MOD_RES (1)..(1): ACETYLATION
MEDHAGTYGLG

SEQ ID NO: 9 - protein, 11 aa, Artificial
  Tau Met11-21
MEDHAGTYGLG

SEQ ID NO: 10 - protein, 21 aa, Artificial
  Tau N-Alpha Acetyl-Met1-21
  MOD_RES (1)..(1): ACETYLATION
MAEPRQEFEVMEDHAGTYGLG

SEQ ID NO: 11 - DNA, 45 bp, Artificial
  Forward primers for Tau-412
cagtgtggtggaattcgccaccatggctgagccccgccaggagtt

SEQ ID NO: 12 - DNA, 44 bp, Artificial
  Forward primers for Met11Tau
cagtgtggtggaattcgccaccatggaagatcacgctgggacgt

SEQ ID NO: 13 - DNA, 39 bp, Artificial
  Reverse primers for Tau412 and  Met11Tau
gatatctgcagaattctcacaaaccctgcttggccaggg

SEQ ID NO: 14 - protein, 12 aa, Artificial
  Tau N-Alpha Acetyl-Met11-21 with a cystein residues to conjugate KLH ((Keyhole limpet hemocyanin)
  MOD_RES (1)..(1): ACETYLATION
MEDHAGTYGLGC